European Patent Specification EP 3 439 462 B1, published May 28, 2025. Title: Increased yield and amount of soluble sugars allocated to fruits in tomato plants. Applicant: VILMORIN & CIE. The sequence listing filed with the application follows.

SEQUENCE LISTING (13 sequences)

SEQ ID NO: 1 - DNA, 121 bp, Lycopersicon esculentum
  Polymorphism (61)..(61): Allele associated with yield increase = T
agaaacaaatacttgttaacaacttaacatgatgtaatggtaaatatgaacacatagaaayggggacaaaaaataaaggtcttctaatgctcttcagatgaagcaacactggtaatgttag

SEQ ID NO: 2 - DNA, 121 bp, Lycopersicon esculentum
  Polymorphism (61)..(61): Allele associated with yield increase = C
gagaaaaagaccattagacaaagaaaaggtgttttgatagctacggagaaaaagagaaagyatagagaaaaaaagcaaaacagggagatgaaaggggtctctaatgggagatccattccct

SEQ ID NO: 3 - DNA, 121 bp, Lycopersicon esculentum
  Polymorphism (61)..(61): Allele associated with yield increase = C
ctggacaatttagagctgaatcttgatattctgccaattgctatggtaattgcagcatcayaagaagctcaaaggcttaaggcttggagatttacttcatggagtggggggagattatggt

SEQ ID NO: 4 - DNA, 121 bp, Lycopersicon esculentum
  Polymorphism (61)..(61): Allele associated with yield increase = G
  misc_feature (62)..(62): n is a, c, g, or t
gtaatagagaaactgaaagaaaaaagggacaaaaatcaagctgtcccggcatttactcttknttttctaccagctttctctacttttgtctgatcttacgaaatgtaaccgcttcactcat

SEQ ID NO: 5 - DNA, 121 bp, Lycopersicon esculentum
  Polymorphism (61)..(61): Allele associated with yield increase = G
tgtctacaaaatgtgggaggtacaaagagggatttgattttagtgctgagagagtgactaraagtattgatgagagcttggagaggctgcagcttgattatgttgatatgttacaatgtca

SEQ ID NO: 6 - DNA, 121 bp, Lycopersicon esculentum
  Polymorphism (61)..(61): Allele associated with yield increase = A
catcaaaatccagaacaaggaaatgaaacgaagcttcttagattgttcttctgaagattgrtccaactattagtttggcctacttacaagttaccgattaacttaagcttaggaagcgaat

SEQ ID NO: 7 - DNA, 121 bp, Lycopersicon esculentum
  Polymorphism (61)..(61): Allele associated with yield increase = G
cacaataaggtaaacatatcatgcagtttgctggttttgactcttagattgagcagacaakagggggttgctgaggtggtaagcactcttcacctccaacaccaaggttgctggtagcaaa

SEQ ID NO: 8 - DNA, 121 bp, Lycopersicon esculentum
  Polymorphism (61)..(61): Allele associated with yield increase = T
actcatcagcaaaaggaacagaatcttggcttctgctcctgtttcttcacccttcacttcyccaaatgaagagtccgaaaaagctaagttagctcaggttgccaaaagactactgaatact

SEQ ID NO: 9 - DNA, 121 bp, Lycopersicon esculentum
  Polymorphism (61)..(61): Allele associated with yield increase = T
cattagagcatctggtggattcagaaattctttcactaaagctcatggaatttcaaacackattggaatcatccttcttctggtatatccagtctgggcattgattctccactttctataa

SEQ ID NO: 10 - DNA, 121 bp, Lycopersicon esculentum
  Polymorphism (61)..(61): Allele associated with yield increase = G
atttgtatttcatcgtagcaagtcagaagtgtatttctgcttgaaatgttttttatgtgcrttgattagtgaaaatacagaatactttctaatggtacacaaaattattttctttgtcgaa

SEQ ID NO: 11 - DNA, 121 bp, Lycopersicon esculentum
  Polymorphism (61)..(61): Allele associated with yield increase = C
tgtaatataatatgcttcaacagtatttattcaacatatagccattgatatcattcaaacmaagcactcccagtttcgcatagaggtaccatttaaccaaactggaggaataaattatctc

SEQ ID NO: 12 - DNA, 121 bp, Lycopersicon esculentum
  Polymorphism (61)..(61): Allele associated with yield increase = A
tcaggaaactcttcttaatctgctattgcggaattatcttcactacaacttgtacgatcamgcagagaaattgaggtcaaaggccccccattttgaagctcattcaaatcagcagttctgc

SEQ ID NO: 13 - DNA, 121 bp, Lycopersicon esculentum
  Polymorphism (61)..(61): Allele associated with yield increase = T
ttttcataggaaaaaattggaggtttacaatgaggtgcttcggaggcttaaagaagaatcygacaataacgacactttacaatctgcttttgacgatgaactttgggctcatttcaatcgc